European Patent Specification EP 3 751 001 B9, published October 4, 2023. Title: Process for preparing ergothioneine. Applicant: NAGASE & CO., LTD. The sequence listing filed with the application follows.

SEQUENCE LISTING (13 sequences)

SEQ ID NO: 1 - DNA, 2322 bp, Schizosaccaromyces pombe
atgaccgaaatcgaaaacatcggtgctctggaagttctgttctctccggaatctatcgaacagtctctgaaacgttgccagctgccgtctaccctgctgtacgacgaaaaaggtctgcgtctgttcgacgaaatcaccaacctgaaagaatactacctgtacgaatctgaactggacatcctgaaaaaattctctgactctatcgctaaccagctgctgtctccggacctgccgaacaccgttatcgaactgggttgcggtaacatgcgtaaaaccaaactgctgctggacgctttcgaaaaaaaaggttgcgacgttcacttctacgctctggacctgaacgaagctgaactgcagaaaggtctgcaggaactgcgtcagaccaccaactaccagcacgttaaagtttctggtatctgcggttgcttcgaacgtctgctgcagtgcctggaccgtttccgttctgaaccgaactctcgtatctctatgctgtacctgggtgcttctatcggtaacttcgaccgtaaatctgctgcttctttcctgcgttctttcgcttctcgtctgaacatccacgacaacctgctgatctctttcgaccaccgtaacaaagctgaactggttcagctggcttacgacgacccgtaccgtatcaccgaaaaattcgaaaaaaacatcctggcttctgttaacgctgttttcggtgaaaacctgttcgacgaaaacgactgggaatacaaatctgtttacgacgaagacctgggtgttcaccgtgcttacctgcaggctaaaaacgaagttaccgttatcaaaggtccgatgttcttccagttcaaaccgtctcacctgatcctgatcgaagaatcttggaaaaactctgaccaggaatgccgtcagatcatcgaaaaaggtgacttcaaactggtttctaaatacgaatctaccatcgctgactactctacctacgttatcaccaaacagttcccggctatgctgcagctgccgctgcagccgtgcccgtctctggctgaatgggacgctctgcgtaaagtttggctgttcatcaccaacaaactgctgaacaaagacaacatgtacaccgcttggattccgctgcgtcacccgccgatcttctacatcggtcacgttccggttttcaacgacatctacctgaccaaaatcgttaaaaacaaagctaccgctaacaaaaaacacttctgggaatggttccagcgtggtatcgacccggacatcgaagacccgtctaaatgccactggcactctgaagttccggaatcttggccgtctccggaccagctgcgtgaatacgaaaaagaatcttgggaataccacatcgttaaactgtgcaaagctatggacgaactgtctacctctgaaaaacgtatcctgtggctgtgctacgaacacgttgctatgcacgttgaaaccaccctgtacatctacgttcagtctttccagaacgctaaccagaccgtttctatctgcggttctctgccggaaccggctgaaaaactgaccaaagctccgctgtgggttaacgttccggaaaccgaaatcgctgttggtatgccgctgaccacccagtacacctctgttggttctaacctgcagtcttctgacctgtctgctcacgaaaacaccgacgaactgttctacttcgcttgggacaacgaaaaaccgatgcgtaaaaaactggtttcttctttctctatcgctaaccgtccgatctctaacggtgaatacctggacttcatcaacaaaaaatctaaaaccgaacgtgtttacccgaaacagtgggctgaaatcgacggtaccctgtacatccgtaccatgtacggtctgctgccgctggacgactacctgggttggccggttatgacctcttacgacgacctgaacaactacgcttcttctcagggttgccgtctgccgaccgaagacgaactgaactgcttctacgaccgtgttctggaacgtaccgacgaaccgtacgtttctaccgaaggtaaagctaccggtttccagcagctgcacccgctggctctgtctgacaactcttctaaccagatcttcaccggtgcttgggaatggacctctaccgttctggaaaaacacgaagacttcgaaccggaagaactgtacccggactacacccgtgacttcttcgacggtaaacacaacgttgttctgggtggttctttcgctaccgctacccgtatctctaaccgtcgttctttccgtaacttctaccaggctggttacaaatacgcttggatcggtgctcgtctggttaaaaactga

SEQ ID NO: 2 - DNA, 1179 bp, Schizosaccaromyces pombe
atggctgaaaacaacgtttacggtcacgaaatgaaaaaacacttcatgctggacccggactacgttaacgttaacaacggttcttgcggtactgaatctctggctgtttacaacaaacacgttcagctgctgaaagaagctcagtctaaaccggacttcatgtgcaacgcttacatgccgatgtacatggaagctacccgtaacgaagttgctaaactgatcggtgctgactcttctaacatcgttttctgcaactctgctaccgacggtatctctaccgttctgctgaccttcccgtgggaacagaacgacgaaatcctgatgctgaacgttgcttacccgacctgcacctacgctgctgacttcgctaaaaaccagcacaacctgcgtctggacgttatcgacgttggtgttgaaatcgacgaagacctgttcctgaaagaagttgaacagcgtttcctgcagtctaaaccgcgtgctttcatctgcgacatcctgtcttctatgccggttatcctgttcccgtgggaaaaagttgttaaactgtgcaaaaaatacaacatcgtttctatcatcgacggtgctcacgctatcggtcacatcccgatgaacctggctaacgttgacccggacttcctgttcaccaacgctcacaaatggctgaactctccggctgcttgcaccgttctgtacgtttctgctaaaaaccacaacctgatcgaagctctgccgctgtcttacggttacggtctgcgtgaaaaagaatctatcgctgttgacaccctgaccaaccgtttcgttaactctttcaaacaggacctgccgaaattcatcgctgttggtgaagctatcaaattccgtaaatctatcggtggtgaagaaaaaatccagcagtactgccacgaaatcgctctgaaaggtgctgaaatcatctctaaagaactgggtacttctttcatcaaaccgccgtacccggttgctatggttaacgttgaagttccgctgcgtaacatcccgtctatcgaaacccagaaagttttctggccgaaatacaacaccttcctgcgtttcatggaattcaaaggtaaattctacacccgtctgtctggtgctgtttacctggaagaatctgacttctactacatcgctaaagttatcaaagacttctgctctctgtga

SEQ ID NO: 3 - DNA, 33 bp, Artificial
  Sp.egt1-Fw primer
aaatagctggtgaatgaccgaaatcgaaaacat

SEQ ID NO: 4 - DNA, 35 bp, Artificial
  Sp.egt1-Rv primer
agccctcctggatcctcagtttttaaccagacgag

SEQ ID NO: 5 - DNA, 27 bp, Artificial
  Sp.egt2-Fw primer
ggatccaggagggctagcatggctgaa

SEQ ID NO: 6 - DNA, 35 bp, Artificial
  Sp.egt2-Rv primer
cgactctagaggatctcacagagagcagaagtctt

SEQ ID NO: 7 - protein, 5 aa, E. coli
SRGRT

SEQ ID NO: 8 - protein, 12 aa, E. coli
  Xaa (2)..(2): Xaa stands for Leu or Ile
  Xaa (5)..(5): Xaa stands for Ile or Val
  Xaa (11)..(11): Xaa stands for Ile or Val
FXARXSRGRTXR

SEQ ID NO: 9 - protein, 33 aa, E. coli
  Xaa (1)..(1): Xaa stands for Glu, Ser or Gly
  Xaa (4)..(4): Xaa stands for Leu, Val or Ser
  Xaa (5)..(5): Xaa stands for Phe or Leu
  Xaa (6)..(6): Xaa stands for Phe or Tyr
  Xaa (8)..(8): Xaa stands for Ala or Gly
  Xaa (11)..(11): Xaa stands for Val, Leu or Ile
  Xaa (12)..(12): Xaa stands for Ala, Ser or Ile
  Xaa (13)..(13): Xaa stands for Trp or Tyr
  Xaa (14)..(14): Xaa stands for Ser or Ala
  Xaa (15)..(15): Xaa stands for Pro or Ile
  Xaa (16)..(16): Xaa stands for Phe or Gln
  Xaa (17)..(17): Xaa stands for Val or Met
  Xaa (18)..(18): Xaa stands for Gly or Ser
  Xaa (19)..(19): Xaa stands for Leu, Met or Ile
  Xaa (21)..(21): Xaa stands for Leu or Ile
  Xaa (24)..(24): Xaa stands for Ile or Val
  Xaa (30)..(30): Xaa stands for Ile or Val
  Xaa (32)..(32): Xaa stands for Gln or Glu
  Xaa (33)..(33): Xaa stands for Phe or Leu
XWTXXXWXWWXXXXXXXXXFXARXSRGRTXRXX

SEQ ID NO: 10 - protein, 677 aa, E. coli
MTDLSHSREKDKINPVVFYTSAGLILLFSLTTILFRDFSALWIGRTLDWVSKTFGWYYLLAATLYIVFVVCIACSRFGSVKLGPEQSKPEFSLLSWAAMLFAAGIGIDLMFFSVAEPVTQYMQPPEGAGQTIEAARQAMVWTLFHYGLTGWSMYALMGMALGYFSYRYNLPLTIRSALYPIFGKRINGPIGHSVDIAAVIGTIFGIATTLGIGVVQLNYGLSVLFDIPDSMAAKAALIALSVIIATISVTSGVDKGIRVLSELNVALALGLILFVLFMGDTSFLLNALVLNVGDYVNRFMGMTLNSFAFDRPVEWMNNWTLFFWAWWVAWSPFVGLFLARISRGRTIRQFVLGTLIIPFTFTLLWLSVFGNSALYEIIHGGAAFAEEAMVHPERGFYSLLAQYPAFTFSASVATITGLLFYVTSADSGALVLGNFTSQLKDINSDAPGWLRVFWSVAIGLLTLGMLMTNGISALQNTTVIMGLPFSFVIFFVMAGLYKSLKVEDYRRESANRDTAPRPLGLQDRLSWKKRLSRLMNYPGTRYTKQMMETVCYPAMEEVAQELRLRGAYVELKSLPPEEGQQLGHLDLLVHMGEEQNFVYQIWPQQYSVPGFTYRARSGKSTYYRLETFLLEGSQGNDLMDYSKEQVITDILDQYERHLNFIHLHREAPGHSVMFPDA

SEQ ID NO: 11 - protein, 504 aa, E. coli
MKNEKRKTGIEPKVFFPPLIIVGILCWLTVRDLDAANVVINAVFSYVTNVWGWAFEWYMVVMLFGWFWLVFGPYAKKRLGNEPPEFSTASWIFMMFASCTSAAVLFWGSIEIYYYISTPPFGLEPNSTGAKELGLAYSLFHWGPLPWATYSFLSVAFAYFFFVRKMEVIRPSSTLVPLVGEKHAKGLFGTIVDNFYLVALIFAMGTSLGLATPLVTECMQWLFGIPHTLQLDAIIITCWIILNAICVACGLQKGVRIASDVRSYLSFLMLGWVFIVSGASFIMNYFTDSVGMLLMYLPRMLFYTDPIAKGGFPQGWTVFYWAWWVIYAIQMSIFLARISRGRTVRELCFGMVLGLTASTWILWTVLGSNTLLLIDKNIINIPNLIEQYGVARAIIETWAALPLSTATMWGFFILCFIATVTLVNACSYTLAMSTCREVRDGEEPPLLVRIGWSILVGIIGIVLLALGGLKPIQTAIIAGGCPLFFVNIMVTLSFIKDAKQNWKD

SEQ ID NO: 12 - DNA, 973 bp, Streptomyces coelicolor
atgagccaattccgcttgacccgcacactgcccgaagatgctaccgatgctgccttacgcgccgatgtactggcgggactgacctccacgcccaaatggttgccgccgaaatggttctatgacgcgcgtgggtcggaactgtttgaagcaatcacggcactgcctgagtactacccaacgcgtgctgaacgcgagattctcgtcgatcgtgcaggggaaattgcggctgccacaggtgcccgcactctcgtggagttgggttcaggcagtagcgagaaaacccgtgtcctcctggatgccctgaccgaacgtaatgggttacgcggctatgtgcctgtggatgtttcggaaagcgcgctggttcaggctggacaggcgttagtggcagaacgtccgggcttacaggtccatgcgctgattgccgacttcactggcggtctgactctgccggacaccccaggtccgcggttagtcgcttttctgggtggcacaattggcaacttactgccgggtgaacgggcagagttcctggcaagcgttcgctcactgctgtctccaggtgatacgcttctgctgggcacggacttggtgaaagacgaaggggttctcgtgcgcgcgtatgatgatgccgcgggagttacgggcgagttcaacaagaacgtactgagcgtggttaatcgcgaactggaagccgactttgccccggcggcgtttgaacacgtagcgttgtggaatgcggaacgggaatggatcgaaatgcgcctgcgttctcgtaccgcccaagcggtgaaaatccaggcactggatctggcagtggactttgccgatggtgaagagttgcgtaccgaggtcagtgcgaagrtttcgccgcgaaggcgtacgcgcagaacttgccgctgccggccttgatctggcgcattggtggaccgatggtggcgaccgttttgcactttccctctcggttgcgcgctaa

SEQ ID NO: 13 - DNA, 1374 bp, Chlorobium limicola
atgcagaacaaaaatttccgtgccccacaaagcgaagccattggcatcctgtacaagctcatagaaactggctccaaacacaaaaacatgtatgaccacacggaaatcaccacagactcactgctggcgctgttaggtagcgaaaaggtcaaaatcattgatgtccgcagtgcggatgcgtataacggttggcgtatgagaggggaggtacgtggtggccatatcaaaggcgcaaaatcgctgccagcgaaatggctcacagatccggaatggttaaacattgtgcgctttaaacagattcgaccagaagatgcgattgtgctctatgggtatacgcctgaagaatgcgaacagactgctactcgctttaaggagaatggctacaacaacgtttcggtgttccatcgctttcatccggattggaccgggaatgatgccttccctatggaccgcttggaacagtacaaccgtttagtgcctgccgaatgggtcaatggtctgatctctggcgaagaaatcccggagtatgacaacgataccttcatcgtgtgtcatgcgcattaccggaatcgtgatgcctaccttagcgggcatattccgggagcaacggacatggacactctggctcttgagtctccggaaacctggaatcgtcgcacaccagaagagctgaaaaaagcgcttgaggaacacggtattaccgcaagcaccaccgtggttctgtacggcaaattcatgcatccggataatgcggatgaatttccgggaagtgctgctggacacataggagcgattcgtctggcgtttatcatgatgtatgcaggcgtggaggatgttcgcgtgttgaatggcggctatcagtcatggacggatgcaggctttgccatcagtaaggatgatgttcccaaaaccaccgtaccggagtttggtgcgccgattccgtcacgtccggaatttgcggtagacattgacgaagctaaagagatgctgcaatcggaagactctgatttggtctgcgttcggtcctatcccgaatacattggggaagtgagcggctacaactatatcaagaaaaaaggtaggattcctggcgccattttcgctgaatgcggttccgatgcataccacatggagaattatcgcaaccatgatcacacgacccgcgagtatcacgaaatcgaggacatttgggccaaaagtgggatcattccgaagaaacatctggccttctactgtggtacgggttggcgtggttcggaagcatggtttaacgcgctactgatgggttggccgcgcgtcagcgtatatgatggtggctggtttgaatggagcaatgaccccgaaaacccgtatgaaaccggcgttccaaaataa